European Patent Specification EP 3 684 416 B1, published March 15, 2023. Title: Novel PSMA-Targeting Amanitin Conjugates. Applicant: Heidelberg Pharma Research GmbH. Application not yet assigned. The sequence listing filed with the application follows.

SEQUENCE LISTING (3 sequences)

SEQ ID NO: 1 - protein, 245 aa, Artificial Sequence
  1
AENLYFQGGGGGEPKSCDKTHTCPPCPAPELLGGPSVFLFPPKPKDTLMISRTPEVTCVVVDVSHEDPEVKFNWYVDGVEVHNAKTKPREEQYASTYRVVSVLTVLHQDWLNGKEYKCKVSNKALPAPIEKTISKAKGQPREPQVYTLPPSRDELTKNQVSLTCLVKGFYPSDIAVEWESNGQPENNYKTTPPVLDSDGSFFLYSKLTVDKSRWQQGNVFSCSVMHEALHNHYTQKSLSLSPGGS

SEQ ID NO: 2 - protein, 6 aa, Artificial Sequence
  2
LPETGG

SEQ ID NO: 3 - protein, 251 aa, Artificial Sequence
  3
AENLYFQGGGGGEPKSCDKTHTCPPCPAPELLGGPSVFLFPPKPKDTLMISRTPEVTCVVVDVSHEDPEVKFNWYVDGVEVHNAKTKPREEQYASTYRVVSVLTVLHQDWLNGKEYKCKVSNKALPAPIEKTISKAKGQPREPQVYTLPPSRDELTKNQVSLTCLVKGFYPSDIAVEWESNGQPENNYKTTPPVLDSDGSFFLYSKLTVDKSRWQQGNVFSCSVMHEALHNHYTQKSLSLSPGGSLPETGG